European Patent Specification EP 3 530 320 B1, published November 15, 2023. Title: Novel IL-4-/IL-13-derived peptide compounds for the treatment or prevention of neurodegenerative or neuroinflammatory diseases. Applicant: Universitätsmedizin der Johannes Gutenberg-Universität Mainz. The sequence listing filed with the application follows.

SEQUENCE LISTING (6 sequences)

SEQ ID NO: 1 - protein, 19 aa, Homo sapiens
WNRSEIIKTGSKTIMREKY

SEQ ID NO: 2 - protein, 27 aa, Homo sapiens
LMRSELIEELVNITGSFVKDLLLHLKK

SEQ ID NO: 3 - protein, 29 aa, Homo sapiens
EIIKTGSRLDRNLWGSGSRAATVLRQFYS

SEQ ID NO: 4 - protein, 19 aa, Mus musculus
RARSEIIGIGSKSIMQMDY

SEQ ID NO: 5 - protein, 27 aa, Mus musculus
LIRSELIEELSNITGSFITKLLSYTKQ

SEQ ID NO: 6 - protein, 29 aa, Mus musculus
EIIGIGPRLFRAFRCSGSRASKVLRIFYL